European Patent Specification EP 3 559 260 B1, published July 3, 2024. Title: Methods and compositions for determining, and for minimizing, the likelihood of development of allergy in infants. Applicant: Murdoch Childrens Research Institute. The sequence listing filed with the application follows.

SEQUENCE LISTING (12 sequences)

SEQ ID NO: 1 - DNA, 253 bp, Prevotella
tacggaaggtccgggcgttatccggatttattgggtttaaagggagcgtaggccggagattaagcgtgttgtgaaatgtagacgctcaacgtctgcactgcagcgcgaactggtttccttgagtacgcacaaagtgggcggaattcgtggtgtagcggtgaaatgcttagatatcacgaagaactccgattgcgaaggcagctcactggagcgcaactgacgctgaagctcgaaagtgcgggtatcgaacagg

SEQ ID NO: 2 - DNA, 253 bp, Prevotella
tacgtatggtgcaagcgttatccggatttattgggtttaaagggagcgtaggccggagattaagcgtgttgtgaaatgtagatgctcaacatctgaactgcagcgcgaactggtttccttgagtacgcacaaagtgggcggaattcgtggtgtagcggtgaaatgcttagatatcacgaagaactccgattgcgaaggcagctcactggagcgcaactgacgctgaagctcgaaagtgcgggtatcgaacagg

SEQ ID NO: 3 - DNA, 21 bp, Prevotella
tacggaaggtccgggcgttat

SEQ ID NO: 4 - DNA, 21 bp, Prevotella
agtgcagacgttgagcgtcta

SEQ ID NO: 5 - DNA, 19 bp, Prevotella
tacgtatggtgcaagcgtt

SEQ ID NO: 6 - DNA, 21 bp, Prevotella
gcagttcagatgttgagcatc

SEQ ID NO: 7 - DNA, 252 bp, Prevotella
tacggaaggtccgggcgttatccggatttattgggtttaaagggagcgtaggccggagattaagcgtgttgtgaaatgtagacgctcaacgtctgcactgcagcgcgaactggtttccttgagtacgcacaaagtgggcggaattcgtggtgtagcggtgaaatgcttagatatcacgaagaactccgattgcgaaggcagctcactggagcgcaactgacgctgaagctcgaaagtgcgggtatcgaacag

SEQ ID NO: 8 - DNA, 1494 bp, Prevotella
  misc_feature (137)..(137): y is c or t
  misc_feature (378)..(378): r is a or g
  misc_feature (1029)..(1029): y is c or t
  misc_feature (1129)..(1129): y is c or t
  misc_feature (1254)..(1254): y is c or t
  misc_feature (1255)..(1255): s is g or c
  misc_feature (1257)..(1257): y is c or t
  misc_feature (1258)..(1258): y is c or t
  misc_feature (1260)..(1260): y is c or t
  misc_feature (1266)..(1266): s is g or c
agagtttgatcctggctcaggatgaacgctagctacaggcttaacacatgcaagtcgaggggaaacgacatcgaaagcttgcttttgatgggcgtcgaccggcgcacgggtgagtaacgcgtatccaacctgcccaycacttggggataaccttgcgaaagtaagactaatacccaatgatatctctagaagacatctgaaagagattaaagatttatcggtgatggatggggatgcgtctgattagcttgttggcggggtaacggcccaccaaggcgacgatcagtaggggttctgagaggaaggtcccccacattggaactgagacacggtccaaactcctacgggaggcagcagtgaggaatattggtcaatggrcgagagcctgaaccagccaagtagcgtgcaggatgacggccctatgggttgtaaactgcttttataagggaataaagtgagcctcgtgaggctttttgcatgtaccttatgaataaggaccggctaattccgtgccagcagccgcggtaatacggaaggtccgggcgttatccggatttattgggtttaaagggagcgtaggccggagattaagcgtgttgtgaaatgtagacgctcaacgtctgcactgcagcgcgaactggtttccttgagtacgcacaaagtgggcggaattcgtggtgtagcggtgaaatgcttagatatcacgaagaactccgattgcgaaggcagctcactggagcgcaactgacgctgaagctcgaaagtgcgggtatcgaacaggattagataccctggtagtccgcacggtaaacgatggatgcccgctgttggtctgaacaggtcagcggccaagcgaaagcattaagcatcccacctggggagtacgccggcaacggtgaaactcaaaggaattgacgggggcccgcacaagcggaggaacatgtggtttaattcgatgatacgcgaggaaaccttacccgggcttgaattgcagaggaaggatttggagacaatgacgcccttcggggyctctgtgaaggtgctgcatggttgtcgtcagctcgtgccgtgaggtgtcggcttaagtgccataacgagcgcaacccctctccttagttgccatcaggtyaagctgggcactctggggacactgccaccgtaaggtgtgaggaaggtggggatgacgtcaaatcagcacggcccttacgtccggggctacacacgtgttacaatggcaggtacagagagacggtyscyygyaaagtsgatcaaatccttaaagcctgtctcagttcggactggggtctgcaacccgaccccacgaagctggattcgctagtaatcgcgcatcagccatggcgcggtgaatacgttcccgggccttgtacacaccgcccgtcaagccatgaaagccgggggcgcctaaagtccgtgaccgtaaggagcggcctagggcgaaactggtaattggggctaagtcgtaacaaggtaacc

SEQ ID NO: 9 - DNA, 1491 bp, Prevotella
  misc_feature (137)..(137): y is c or t
  misc_feature (378)..(378): r is a or g
  misc_feature (385)..(385): y is c or t
  misc_feature (412)..(412): w is a or t
  misc_feature (469)..(469): r is a or g
  misc_feature (1126)..(1126): y is c or t
  misc_feature (1128)..(1128): w is a or t
  misc_feature (1195)..(1195): y is c or t
  misc_feature (1251)..(1251): y is c or t
  misc_feature (1252)..(1252): s is g or c
  misc_feature (1253)..(1253): y is c or t
  misc_feature (1254)..(1254): w is a or t
  misc_feature (1255)..(1255): y is c or t
  misc_feature (1257)..(1257): y is c or t
  misc_feature (1260)..(1260): r is a or g
  misc_feature (1261)..(1261): w is a or t
  misc_feature (1263)..(1263): s is g or c
agagtttgatcctggctcaggatgaacgctagctacaggcttaacacatgcaagtcgaggggaaacgacatcgaaagcttgcttttgatgggcgtcgaccggcgcacgggtgagtaacgcgtatccaacctgcccaycacttggggataaccttgcgaaagtaagactaatacccaatgatatctctagaagacatctgaaagagattaaagatttatcggtgatggatggggatgcgtctgattagcttgttggcggggtaacggcccaccaaggcgacgatcagtaggggttctgagaggaaggtcccccacattggaactgagacacggtccaaactcctacgggaggcagcagtgaggaatattggtcaatggrcgagagyctgaaccagccaagtagcgtgcaggawgacggccctatgggttgtaaactgcttttataagggaataaagtgagcctcgtgagrctttttgcatgtaccttatgaataaggaccggctaattccgtgccagcagccgcggtaatacggaaggtccgggcgttatccggatttattgggtttaaagggagcgtaggccggagattaagcgtgttgtgaaatgtagacgctcaacgtctgcactgcagcgcgaactggtttccttgagtacgcacaaagtgggcggaattcgtggtgtagcggtgaaatgcttagatatcacgaagaactccgattgcgaaggcagctcactggagcgcaactgacgctgaagctcgaaagtgcgggtatcgaacaggattagataccctggtagtccgcacggtaaacgatggatgcccgctgttggtctgaacaggtcagcggccaagcgaaagcattaagcatcccacctgggggagtacgccggcaacggtgaaactcaaaggaattgacggggcccgcacaagcggaggaacatgtggttaattcgatgatacgcgaggaaccttacccgggcttgaattgcagaggaaggattggagacaatgacgcccttcggggcctctgtgaaggtgctgcatggttgtcgtcagctcgtgccgtgaggtgtcggcttaagtgccataacgagcgcaacccctctccttagttgccatcaggtyawgctgggcactctggggacactgccaccgtaaggtgtgaggaaggtggggatgacgtcaaatcagcayggcccttacgtccggggctacacacgtgttacaatggcaggtacagagagacggtysywygyaarwtsgatcaaatccttaaagcctgtctcagttcggactggggtctgcaacccgaccccacgaagctggattcgctagtaatcgcgcatcagccatggcgcggtgaatacgttcccgggccttgtacacaccgcccgtcaagccatgaaagccgggggcgcctaaagtccgtgaccgtaaggagcggcctagggcgaaactggtaattggggctaagtcgtaacaaggtaacc

SEQ ID NO: 10 - DNA, 1493 bp, Prevotella
  misc_feature (378)..(378): r is a or g
  misc_feature (385)..(385): y is c or t
  misc_feature (412)..(412): w is a or t
  misc_feature (469)..(469): r is a or g
  misc_feature (1028)..(1028): y is c or t
  misc_feature (1038)..(1038): n is a, c, g, or t
  misc_feature (1253)..(1253): y is c or t
  misc_feature (1254)..(1254): s is g or c
  misc_feature (1255)..(1255): y is c or t
  misc_feature (1256)..(1256): w is a or t
  misc_feature (1259)..(1259): y is c or t
  misc_feature (1262)..(1262): r is a or g
  misc_feature (1263)..(1263): w is a or t
  misc_feature (1265)..(1265): s is g or c
agagtttgatcctggctcaggatgaacgctagctacaggcttaacacatgcaagtcgaggggaaacgacatcgaaagcttgcttttgatgggcgtcgaccggcgcacgggtgagtaacgcgtatccaacctgcccaccacttggggataaccttgcgaaagtaagactaatacccaatgatatctctagaagacatctgaaagagattaaagatttatcggtgatggatggggatgcgtctgattagcttgttggcggggtaacggcccaccaaggcgacgatcagtaggggttctgagaggaaggtcccccacattggaactgagacacggtccaaactcctacgggaggcagcagtgaggaatattggtcaatggrcgagagyctgaaccagccaagtagcgtgcaggawgacggccctatgggttgtaaactgcttttataagggaataaagtgagcctcgtgagrctttttgcatgtaccttatgaataaggaccggctaattccgtgccagcagccgcggtaatacggaaggtccgggcgttatccggatttattgggtttaaagggagcgtaggccggagattaagcgtgttgtgaaatgtagacgctcaacgtctgcactgcagcgcgaactggtttccttgagtacgcacaaagtgggcggaattcgtggtgtagcggtgaaatgcttagatatcacgaagaactccgattgcgaaggcagctcactggagcgcaactgacgctgaagctcgaaagtgcgggtatcgaacaggattagataccctggtagtccgcacggtaaacgatggatgcccgctgttggtctgaacaggtcagcggccaagcgaaagcattaagcatcccacctggggagtacgccggcaacggtgaaactcaaaggaattgacgggggcccgcacaagcggaggaacatgtggtttaattcgatgatacgcgaggaaccttacccgggcttgaattgcagaggaaggatttggagacaatgacgcccttcggggyctctgtgaangtgctgcatggttgtcgtcagctcgtgccgtgaggtgtcggcttaagtgccataacgagcgcaacccctctccttagttgccatcaggtcaagctgggcactctggggacactgccaccgtaaggtgtgaggaaggtggggatgacgtcaaatcagcacggcccttacgtccggggctacacacgtgttacaatggcaggtacagagagacggtysywtgyaarwtsgatcaaatccttaaagcctgtctcagttcggactggggtctgcaacccgaccccacgaagctggattcgctagtaatcgcgcatcagccatggcgcggtgaatacgttcccgggccttgtacacaccgcccgtcaagccatgaaagccgggggcgcctaaagtccgtgaccgtaaggagcggcctagggcgaaactggtaattggggctaagtcgtaacaaggtaacc

SEQ ID NO: 11 - DNA, 1493 bp, Prevotella
  misc_feature (137)..(137): y is c or t
  misc_feature (378)..(378): r is a or g
  misc_feature (385)..(385): y is c or t
  misc_feature (469)..(469): r is a or g
  misc_feature (1028)..(1028): y is c or t
  misc_feature (1128)..(1128): y is c or t
  misc_feature (1253)..(1253): y is c or t
  misc_feature (1254)..(1254): s is g or c
  misc_feature (1255)..(1255): y is c or t
  misc_feature (1256)..(1256): w is a or t
  misc_feature (1257)..(1257): y is c or t
  misc_feature (1259)..(1259): y is c or t
  misc_feature (1262)..(1262): r is a or g
  misc_feature (1263)..(1263): w is a or t
  misc_feature (1265)..(1265): s is g or c
agagtttgatcctggctcaggatgaacgctagctacaggcttaacacatgcaagtcgaggggaaacgacatcgaaagcttgcttttgatgggcgtcgaccggcgcacgggtgagtaacgcgtatccaacctgcccaycacttggggataaccttgcgaaagtaagactaatacccaatgatatctctagaagacatctgaaagagattaaagatttatcggtgatggatggggatgcgtctgattagcttgttggcggggtaacggcccaccaaggcgacgatcagtaggggttctgagaggaaggtcccccacattggaactgagacacggtccaaactcctacgggaggcagcagtgaggaatattggtcaatggrcgagagyctgaaccagccaagtagcgtgcaggatgacggccctatgggttgtaaactgcttttataagggaataaagtgagcctcgtgagrctttttgcatgtaccttatgaataaggaccggctaattccgtgccagcagccgcggtaatacggaaggtccgggcgttatccggatttattgggtttaaagggagcgtaggccggagattaagcgtgttgtgaaatgtagacgctcaacgtctgcactgcagcgcgaactggtttccttgagtacgcacaaagtgggcggaattcgtggtgtagcggtgaaatgcttagatatcacgaagaactccgattgcgaaggcagctcactggagcgcaactgacgctgaagctcgaaagtgcgggtatcgaacaggattagataccctggtagtccgcacggtaaacgatggatgcccgctgttggtctgaacaggtcagcggccaagcgaaagcattaagcatcccacctggggagtacgccggcaacggtgaaactcaaaggaattgacgggggcccgcacaagcggaggaacatgtggtttaattcgatgatacgcgaggaaccttacccgggcttgaattgcagaggaaggatttggagacaatgacgcccttcggggyctctgtgaaggtgctgcatggttgtcgtcagctcgtgccgtgaggtgtcggcttaagtgccataacgagcgcaacccctctccttagttgccatcaggtyaagctgggcactctggggacactgccaccgtaaggtgtgaggaaggtggggatgacgtcaaatcagcacggcccttacgtccggggctacacacgtgttacaatggcaggtacagagagacggtysywygyaarwtsgatcaaatccttaaagcctgtctcagttcggactggggtctgcaacccgaccccacgaagctggattcgctagtaatcgcgcatcagccatggcgcggtgaatacgttcccgggccttgtacacaccgcccgtcaagccatgaaagccgggggcgcctaaagtccgtgaccgtaaggagcggcctagggcgaaactggtaattggggctaagtcgtaacaaggtaacc

SEQ ID NO: 12 - DNA, 1493 bp, Prevotella
  misc_feature (378)..(378): r is a or g
  misc_feature (385)..(385): y is c or t
  misc_feature (412)..(412): w is a or t
  misc_feature (460)..(460): y is c or t
  misc_feature (469)..(469): r is a or g
  misc_feature (1128)..(1128): y is c or t
  misc_feature (1253)..(1253): y is c or t
  misc_feature (1254)..(1254): s is g or c
  misc_feature (1255)..(1255): y is c or t
  misc_feature (1256)..(1256): w is a or t
  misc_feature (1259)..(1259): y is c or t
  misc_feature (1262)..(1262): r is a or g
  misc_feature (1263)..(1264): w is a or t
  misc_feature (1265)..(1265): s is g or c
agagtttgatcctggctcaggatgaacgctagctacaggcttaacacatgcaagtcgaggggaaacgacatcgaaagcttgcttttgatgggcgtcgaccggcgcacgggtgagtaacgcgtatccaacctgcccaccacttggggataaccttgcgaaagtaagactaatacccaatgatatctctagaagacatctgaaagagattaaagatttatcggtgatggatggggatgcgtctgattagcttgttggcggggtaacggcccaccaaggcgacgatcagtaggggttctgagaggaaggtcccccacattggaactgagacacggtccaaactcctacgggaggcagcagtgaggaatattggtcaatggrcgagagyctgaaccagccaagtagcgtgcaggawgacggccctatgggttgtaaactgcttttataagggaataaagtgagyctcgtgagrctttttgcatgtaccttatgaataaggaccggctaattccgtgccagcagccgcggtaatacggaaggtccgggcgttatccggatttattgggtttaaagggagcgtaggccggagattaagcgtgttgtgaaatgtagacgctcaacgtctgcactgcagcgcgaactggtttccttgagtacgcacaaagtgggcggaattcgtggtgtagcggtgaaatgcttagatatcacgaagaactccgattgcgaaggcagctcactggagcgcaactgacgctgaagctcgaaagtgcgggtatcgaacaggattagataccctggtagtccgcacggtaaacgatggatgcccgctgttggtctgaacaggtcagcggccaagcgaaagcattaagcatcccacctggggagtacgccggcaacggtgaaactcaaaggaattgacgggggcccgcacaagcggaggaacatgtggtttaattcgatgatacgcgaggaaccttacccgggcttgaattgcagaggaaggatttggagacaatgacgcccttcggggcctctgtgaaggtgctgcatggttgtcgtcagctcgtgccgtgaggtgtcggcttaagtgccataacgagcgcaacccctctccttagttgccatcaggtyaagctgggcactctggggacactgccaccgtaaggtgtgaggaaggtggggatgacgtcaaatcagcacggcccttacgtccggggctacacacgtgttacaatggcaggtacagagagacggtysywtgyaarwwsgatcaaatccttaaagcctgtctcagttcggactggggtctgcaacccgaccccacgaagctggattcgctagtaatcgcgcatcagccatggcgcggtgaatacgttcccgggccttgtacacaccgcccgtcaagccatgaaagccgggggcgcctaaagtccgtgaccgtaaggagcggcctagggcgaaactggtaattggggctaagtcgtaacaaggtaacc